European Patent Application EP 4 667 498 A1, published December 24, 2025. Title: GLP-1类似物-Fc融合蛋白及其应用. Applicant: 张菁. Application CN. The sequence listing filed with the application follows.

SEQUENCE LISTING (8 sequences)

SEQ ID NO: 1 - protein, 31 aa, synthetic construct
HAEGTFTSDVSSYLEGQAAKEFIAWLVKGRG

SEQ ID NO: 2 - protein, 31 aa, synthetic construct
HGEGTFPSDVSSYLEGQAAKEFIAWLVKGRG

SEQ ID NO: 3 - protein, 227 aa, synthetic construct
SKYGPPCPPCPAPEAAGGPSVFLFPPKPKDTLMISRTPEVTCVVVDVSQEDPEVQFNWYVDGVEVHNAKTKPREEQFNSTYRVVSVLTVLHQDWLNGKEYKCKVSNKGLPSSIEKTISKAKGQPREPQVYTLPPSQEEMTKNQVSLTCLVKGFYPSDIAVEWESNGQPENNYKTTPPVLDSDGSFFLYSRLTVDKSRWQEGNVFSCSVMHEALHNHYTQKSLSLSLG

SEQ ID NO: 4 - protein, 5 aa, synthetic construct
GGGGS

SEQ ID NO: 5 - protein, 19 aa, synthetic construct
GGGGGGSGGGGSGGGGSAE

SEQ ID NO: 6 - protein, 299 aa, synthetic construct
MDMRVPAQLLGLLLLWFPGSRCHGEGTFPSDVSSYLEGQAAKEFIAWLVKGRGGGGGGGSGGGGSGGGGSAESKYGPPCPPCPAPEAAGGPSVFLFPPKPKDTLMISRTPEVTCVVVDVSQEDPEVQFNWYVDGVEVHNAKTKPREEQFNSTYRVVSVLTVLHQDWLNGKEYKCKVSNKGLPSSIEKTISKAKGQPREPQVYTLPPSQEEMTKNQVSLTCLVKGFYPSDIAVEWESNGQPENNYKTTPPVLDSDGSFFLYSRLTVDKSRWQEGNVFSCSVMHEALHNHYTQKSLSLSLG

SEQ ID NO: 7 - protein, 277 aa, synthetic construct
HGEGTFPSDVSSYLEGQAAKEFIAWLVKGRGGGGGGGSGGGGSGGGGSAESKYGPPCPPCPAPEAAGGPSVFLFPPKPKDTLMISRTPEVTCVVVDVSQEDPEVQFNWYVDGVEVHNAKTKPREEQFNSTYRVVSVLTVLHQDWLNGKEYKCKVSNKGLPSSIEKTISKAKGQPREPQVYTLPPSQEEMTKNQVSLTCLVKGFYPSDIAVEWESNGQPENNYKTTPPVLDSDGSFFLYSRLTVDKSRWQEGNVFSCSVMHEALHNHYTQKSLSLSLG

SEQ ID NO: 8 - DNA, 897 bp, synthetic construct
  source 1..897: mol_type = other DNA
atggacatgcgcgtgcccgcccagctgctgggcctgctgctgctgtggttccccggatcccgatgccatggtgaaggtacttttccaagtgatgtgagctcctacctggaaggccaggccgctaaagagttcatcgcttggctcgtcaagggcagaggcggaggcggaggaggtggctccggcggcggcggctctggcggcggcggatctgccgagagcaagtacggccccccatgtcctccttgccctgctcctgaggccgctggcggcccttccgtgtttctgttccctcccaagccaaaggacaccctgatgatctctcggacccctgaagtcacatgcgtggtggtggacgtgtctcaagaggatcccgaggtgcagtttaactggtacgtggatggcgtggaagtgcacaacgccaagaccaagcccagagaggaacagttcaactccacctacagagtcgtttctgtgctgaccgtgctgcaccaggactggctgaacggcaaagagtacaagtgcaaagtgtccaataagggcctgcctagctccatcgagaagaccatctccaaggccaagggacagcctagagaacctcaagtgtacacactgcctccttctcaggaagagatgaccaagaaccaggtgagcctgacctgtctggtgaagggcttctacccctccgacatcgccgtggaatgggagtctaatggccagcctgagaacaactacaaaaccaccccacctgtgctggattctgacggctctttcttcctgtacagccggctgaccgtggacaagtcccggtggcaggagggcaacgtgttctcctgctccgtgatgcacgaggccctgcataaccactatacacagaagtccctgtccctgtctttgggc